European Patent Application EP 4 603 509 A1, published August 20, 2025. Title: MULTIFUNCTIONAL RECOMBINANT ANTIBODY, AND PREPARATION METHOD AND USE THEREOF. Applicant: SHENZHEN BAISHITONG TECHNOLOGY DEVELOPMENT COMPANY LIMITED. The sequence listing filed with the application follows.

SEQUENCE LISTING (31 sequences)

SEQ ID NO: 1 - protein, 227 aa, Artificial sequence
LEVQVPEDPVVALVGTDATLCCSFSPEPGFSLAQLNLIWQLTDTKQLVHSFAEGQDQGSAYANRTALFPDLLAQGNASLRLQRVRVADEGSFTCFVSIRDFGSAAVSLQVAAPYSKPSMTLEPNKDLRPGDTVTITCSSYQGYPEAEVFWQDGQGVPLTGNVTTSQMANEQGLFDVHSILRVVLGANGTYSCLVRNPVLQQDAHSSVTITPQRSPTGAVEVQVPEDP

SEQ ID NO: 2 - protein, 437 aa, Artificial sequence
LEVQVPEDPVVALVGTDATLRCSFSPEPGFSLAQLNLIWQLTDTKQLVHSFTEGRDQGSAYANRTALFLDLLAQGNASLRLQRVRVADEGSFTCFVSIRDFGSAAVSLQVAAPYSKPSMTLEPNKDLRPGDTVTITCSSYRGYPEAEVFWQDGQGAPLTGNVTTSQMANEQGLFDVHSVLRVVLGANGTYSCLVRNPVLQQDAHGSITITPQRSPTGAVEVQVPEDPVVALVGTDATLRCSFSPEPGFSLAQLNLIWQLTDTKQLVHSFTEGRDQGSAYANRTALFLDLLAQGNASLRLQRVRVADEGSFTCFVSIRDFGSAAVSLQVAAPYSKPSMTLEPNKDLRPGDTVTITCSSYRGYPEAEVFWQDGQGAPLTGNVTTSQMANEQGLFDVHSVLRVVLGANGTYSCLVRNPVLQQDAHGSITITPQRSPTGFF

SEQ ID NO: 3 - protein, 216 aa, Artificial sequence
VEVQVSEDPVVALVDTDATLRCSFSPEPGFSLAQLNLIWQLTDTKQLVHSFTEGRDQGSAYSNRTALFPDLLVQGNASLRLQRVRVTDEGSYTCFVSIQDFDSAAVSLQVAAPYSKPSMTLEPNKDLRPGNMVTITCSSYQGYPEAEVFWKDGQGVPLTGNVTTSQMANERGLFDVHSVLRVVLGANGTYSCLVRNPVLQQDAHGSVTITGQPLTF

SEQ ID NO: 4 - protein, 366 aa, Artificial sequence
CAGGTCCAGCTGAAACAGTCTGGAATTGAGCTGGTGAGGCCTGGGGCTTCAGTGAAGCTGTCCTGCAAGACTTCTGGATACATCTTCACCGCCGACTGGATTTACTGGGTAAAACAGAGGTCTGGTCAGGGCCTTGAGTGGATTGGAAGGATTTATCCTGGAGTTGATAGTACTTACTACAATGAGAAATTCAAGGACAAGGCCATACTGACTGCAGACAAATCCTCCAGCACTGCCTACATGCAACTCAACAGCCTGAAATCTGAGGACTCTGCTGTCTATTTCTGTGCGCGAGGGGGAGAGGTACGACGGGATTTCTATGCTTTGGACTACTGGGGTCAAGGAACCTCAGTCACCGTCTCCTCA

SEQ ID NO: 5 - protein, 122 aa, Artificial sequence
QVQLKQSGIELVRPGASVKLSCKTSGYIFTADWIYWVKQRSGQGLEWIGRIYPGVDSTYYNEKFKDKAILTADKSSSTAYMQLNSLKSEDSAVYFCARGGEVRRDFYALDYWGQGTSVTVSS

SEQ ID NO: 6 - protein, 321 aa, Artificial sequence
AACATTGTTATGACCCAATCTCCCGAATCCATGTCCATGTCACTTGGAGAGAGGGTCACCTTGAGCTGCAAGGCCAGTGAGAATGTGGGTACTTATGTATCCTGGTATCAACAGAAACCAGAGCAGTCTCCTAAATTGCTGATATACGGGGCATCCAACCGGTACACTGGGGTCCCCGCTCGCTTCACAGGCAGTGGATCTGCAACAGATTTCACTCTGACCATCAGCAGTGTGCAGGCTGAAGACCTTGCAGATTATCACTGTGGACAGAGGTACAGCTATCCATTCACGTTCGGCTCGGGGACAAAGTTGGAAATAAAA

SEQ ID NO: 7 - protein, 107 aa, Artificial sequence
NIVMTQSPESMSMSLGERVTLSCKASENVGTYVSWYQQKPEQSPKLLIYGASNRYTGVPARFTGSGSATDFTLTISSVQAEDLADYHCGQRYSYPFTFGSGTKLEIK

SEQ ID NO: 8 - protein, 330 aa, Artificial sequence [sequence omitted]

SEQ ID NO: 9 - protein, 107 aa, Artificial sequence [sequence omitted]

SEQ ID NO: 10 - protein, 8 aa, Artificial sequence
KTSGYIFT

SEQ ID NO: 11 - protein, 6 aa, Artificial sequence
IGRIYP

SEQ ID NO: 12 - protein, 15 aa, Artificial sequence
ARGGEVRRDFYALDY

SEQ ID NO: 13 - protein, 9 aa, Artificial sequence
KASENVGTY

SEQ ID NO: 14 - protein, 7 aa, Artificial sequence
GASNRYT

SEQ ID NO: 15 - protein, 9 aa, Artificial sequence
GQRYSYPFT

SEQ ID NO: 16 - protein, 111 aa, Artificial sequence
LEVQVPEDPVVALVGTDATLCCSFSPEPGFSLAQLNLIWQLTDTKQLVHSFAEGQDQGSAYANRTALFPDLLAQGNASLRLQRVRVADEGSFTCFVSIRDFGSAAVSLQVA

SEQ ID NO: 17 - protein, 94 aa, Artificial sequence
PSMTLEPNKDLRPGDTVTITCSSYQGYPEAEVFWQDGQGVPLTGNVTTSQMANEQGLFDVHSILRVVLGANGTYSCLVRNPVLQQDAHSSVTIT

SEQ ID NO: 18 - protein, 232 aa, Artificial sequence
EPKSCDKTHTCPPCPAPELLGGPSVFLFPPKPKDTLMISRTPEVTCVVVDVSHEDPEVKFNWYVDGVEVHNAKTKPREEQYNSTYRVVSVLTVLHQDWLNGKEYKCKVSNKALPAPIEKTISKAKGQPREPQVYTLPPSRDELTKNQVSLTCLVKGFYPSDIAVEWESNGQPENNYKTTPPVLDSDGSFFLYSKLTVDKSRWQQGNVFSCSVMHEALHNHYTQKSLSLSPGK

SEQ ID NO: 19 - protein, 343 aa, Artificial sequence
LEVQVPEDPVVALVGTDATLCCSFSPEPGFSLAQLNLIWQLTDTKQLVHSFAEGQDQGSAYANRTALFPDLLAQGNASLRLQRVRVADEGSFTCFVSIRDFGSAAVSLQVAEPKSCDKTHTCPPCPAPELLGGPSVFLFPPKPKDTLMISRTPEVTCVVVDVSHEDPEVKFNWYVDGVEVHNAKTKPREEQYNSTYRVVSVLTVLHQDWLNGKEYKCKVSNKALPAPIEKTISKAKGQPREPQVYTLPPSRDELTKNQVSLTCLVKGFYPSDIAVEWESNGQPENNYKTTPPVLDSDGSFFLYSKLTVDKSRWQQGNVFSCSVMHEALHNHYTQKSLSLSPGK

SEQ ID NO: 20 - protein, 326 aa, Artificial sequence
PSMTLEPNKDLRPGDTVTITCSSYQGYPEAEVFWQDGQGVPLTGNVTTSQMANEQGLFDVHSILRVVLGANGTYSCLVRNPVLQQDAHSSVTITEPKSCDKTHTCPPCPAPELLGGPSVFLFPPKPKDTLMISRTPEVTCVVVDVSHEDPEVKFNWYVDGVEVHNAKTKPREEQYNSTYRVVSVLTVLHQDWLNGKEYKCKVSNKALPAPIEKTISKAKGQPREPQVYTLPPSRDELTKNQVSLTCLVKGFYPSDIAVEWESNGQPENNYKTTPPVLDSDGSFFLYSKLTVDKSRWQQGNVFSCSVMHEALHNHYTQKSLSLSPGK

SEQ ID NO: 21 - protein, 122 aa, Artificial sequence
QVQLVQSGAEVKKPGSSVKVSCKASGYIFTADWIYWVRQAPGQGLEWMGRIYPGVDTTYYAQKFQGRVTITADKSTSTAYMELSSLRSEDTAVYYCARGGEVRRDFYALDYWGQGTTVTVSS

SEQ ID NO: 22 - protein, 107 aa, Artificial sequence
EIVMTQSPPTLSLSPGERVTLSCRASENVGTYVSWYQQKPGQAPRLLIYGASNRYTGIPARFSGSGSGTDFTLTISSLQPEDFAVYYCGQRYSYPFTFGGGTKLEIK

SEQ ID NO: 23 - protein, 452 aa, Artificial sequence
QVQLVQSGAEVKKPGSSVKVSCKASGYIFTADWIYWVRQAPGQGLEWMGRIYPGVDTTYYAQKFQGRVTITADKSTSTAYMELSSLRSEDTAVYYCARGGEVRRDFYALDYWGQGTTVTVSSASTKGPSVFPLAPSSKSTSGGTAALGCLVKDYFPEPVTVSWNSGALTSGVHTFPAVLQSSGLYSLSSVVTVPSSSLGTQTYICNVNHKPSNTKVDKKVEPKSCDKTHTCPPCPAPELLGGPSVFLFPPKPKDTLMISRTPEVTCVVVDVSHEDPEVKFNWYVDGVEVHNAKTKPREEQYNSTYRVVSVLTVLHQDWLNGKEYKCKVSNKALPAPIEKTISKAKGQPREPQVYTLPPSRDELTKNQVSLTCLVKGFYPSDIAVEWESNGQPENNYKTTPPVLDSDGSFFLYSKLTVDKSRWQQGNVFSCSVMHEALHNHYTQKSLSLSPGK

SEQ ID NO: 24 - protein, 214 aa, Artificial sequence
EIVMTQSPPTLSLSPGERVTLSCRASENVGTYVSWYQQKPGQAPRLLIYGASNRYTGIPARFSGSGSGTDFTLTISSLQPEDFAVYYCGQRYSYPFTFGGGTKLEIKRTVAAPSVFIFPPSDEQLKSGTASVVCLLNNFYPREAKVQWKVDNALQSGNSQESVTEQDSKDSTYSLSSTLTLSKADYEKHKVYACEVTHQGLSSPVTKSFNRGEC

SEQ ID NO: 25 - protein, 330 aa, Artificial sequence
ASTKGPSVFPLAPSSKSTSGGTAALGCLVKDYFPEPVTVSWNSGALTSGVHTFPAVLQSSGLYSLSSVVTVPSSSLGTQTYICNVNHKPSNTKVDKKVEPKSCDKTHTCPPCPAPELLGGPSVFLFPPKPKDTLMISRTPEVTCVVVDVSHEDPEVKFNWYVDGVEVHNAKTKPREEQYNSTYRVVSVLTVLAQDWLNGKEYKCKVSNKALPAPIEKTISKAKGQPREPQVYTLPPSRDELTKNQVSLTCLVKGFYPSDIAVEWESNGQPENNYKTTPPVLDSDGSFFLYSKLTVDKSRWQQGNVFSCSVMHEALHNQYTQKSLSLSPGK

SEQ ID NO: 26 - protein, 452 aa, Artificial sequence
QVQLVQSGAEVKKPGSSVKVSCKASGYIFTADWIYWVRQAPGQGLEWMGRIYPGVDTTYYAQKFQGRVTITADKSTSTAYMELSSLRSEDTAVYYCARGGEVRRDFYALDYWGQGTTVTVSSASTKGPSVFPLAPSSKSTSGGTAALGCLVKDYFPEPVTVSWNSGALTSGVHTFPAVLQSSGLYSLSSVVTVPSSSLGTQTYICNVNHKPSNTKVDKKVEPKSCDKTHTCPPCPAPELLGGPSVFLFPPKPKDTLMISRTPEVTCVVVDVSHEDPEVKFNWYVDGVEVHNAKTKPREEQYNSTYRVVSVLTVLAQDWLNGKEYKCKVSNKALPAPIEKTISKAKGQPREPQVYTLPPSRDELTKNQVSLTCLVKGFYPSDIAVEWESNGQPENNYKTTPPVLDSDGSFFLYSKLTVDKSRWQQGNVFSCSVMHEALHNQYTQKSLSLSPGK

SEQ ID NO: 27 - protein, 65 aa, Artificial sequence
ITCPPPMSVEHADIWVKSYSLYSRERYICNSGFKRKAGTSSLTECVLNKATNVAHWTTPSLKCIR

SEQ ID NO: 28 - protein, 114 aa, Artificial sequence
NWVNVISDLKKIEDLIQSMHIDATLYTESDVHPSCKVTAMKCFLLELQVISLESGDASIHDTVENLIILANDSLSSNGNVTESGCKECEELEEKNIKEFLQSFVHIVQMFINTS

SEQ ID NO: 29 - protein, 209 aa, Artificial sequence
ITCPPPMSVEHADIWVKSYSLYSRERYICNSGFKRKAGTSSLTECVLNKATNVAHWTTPSLKCIRGGGGSGGGGSGGGGSGGGGSGGGGSGGGGSNWVNVISDLKKIEDLIQSMHIDATLYTESDVHPSCKVTAMKCFLLELQVISLESGDASIHDTVENLIILANDSLSSNGNVTESGCKECEELEEKNIKEFLQSFVHIVQMFINTS

SEQ ID NO: 30 - protein, 676 aa, Artificial sequence
QVQLVQSGAEVKKPGSSVKVSCKASGYIFTADWIYWVRQAPGQGLEWMGRIYPGVDTTYYAQKFQGRVTITADKSTSTAYMELSSLRSEDTAVYYCARGGEVRRDFYALDYWGQGTTVTVSSASTKGPSVFPLAPSSKSTSGGTAALGCLVKDYFPEPVTVSWNSGALTSGVHTFPAVLQSSGLYSLSSVVTVPSSSLGTQTYICNVNHKPSNTKVDKKVEPKSCDKTHTCPPCPAPELLGGPSVFLFPPKPKDTLMISRTPEVTCVVVDVSHEDPEVKFNWYVDGVEVHNAKTKPREEQYNSTYRVVSVLTVLHQDWLNGKEYKCKVSNKALPAPIEKTISKAKGQPREPQVYTLPPSRDELTKNQVSLTCLVKGFYPSDIAVEWESNGQPENNYKTTPPVLDSDGSFFLYSKLTVDKSRWQQGNVFSCSVMHEALHNHYTQKSLSLSPGKGGGGSGGGGSGGGGSITCPPPMSVEHADIWVKSYSLYSRERYICNSGFKRKAGTSSLTECVLNKATNVAHWTTPSLKCIRGGGGSGGGGSGGGGSGGGGSGGGGSGGGGSNWVNVISDLKKIEDLIQSMHIDATLYTESDVHPSCKVTAMKCFLLELQVISLESGDASIHDTVENLIILANDSLSSNGNVTESGCKECEELEEKNIKEFLQSFVHIVQMFINTS

SEQ ID NO: 31 - protein, 676 aa, Artificial sequence
QVQLVQSGAEVKKPGSSVKVSCKASGYIFTADWIYWVRQAPGQGLEWMGRIYPGVDTTYYAQKFQGRVTITADKSTSTAYMELSSLRSEDTAVYYCARGGEVRRDFYALDYWGQGTTVTVSSASTKGPSVFPLAPSSKSTSGGTAALGCLVKDYFPEPVTVSWNSGALTSGVHTFPAVLQSSGLYSLSSVVTVPSSSLGTQTYICNVNHKPSNTKVDKKVEPKSCDKTHTCPPCPAPELLGGPSVFLFPPKPKDTLMISRTPEVTCVVVDVSHEDPEVKFNWYVDGVEVHNAKTKPREEQYNSTYRVVSVLTVLAQDWLNGKEYKCKVSNKALPAPIEKTISKAKGQPREPQVYTLPPSRDELTKNQVSLTCLVKGFYPSDIAVEWESNGQPENNYKTTPPVLDSDGSFFLYSKLTVDKSRWQQGNVFSCSVMHEALHNQYTQKSLSLSPGKGGGGSGGGGSGGGGSITCPPPMSVEHADIWVKSYSLYSRERYICNSGFKRKAGTSSLTECVLNKATNVAHWTTPSLKCIRGGGGSGGGGSGGGGSGGGGSGGGGSGGGGSNWVNVISDLKKIEDLIQSMHIDATLYTESDVHPSCKVTAMKCFLLELQVISLESGDASIHDTVENLIILANDSLSSNGNVTESGCKECEELEEKNIKEFLQSFVHIVQMFINTS